European Patent Specification EP 3 757 115 B1, published July 9, 2025. Title: Proteins with Diagnostic and Terapeutic Uses. Applicant: The University Court of the University of Edinburgh. The sequence listing filed with the application follows.

SEQUENCE LISTING (9 sequences)

SEQ ID NO: 1 - protein, 104 aa, Streptococcus pneumoniae
ATENEGSTQAATSSNMAKTEHRKAAKQVVDEYIEKMLREIQLDRRKHTQNVALNIKLSAIKTKYLRELNVLEEKSKDELPSEIKAKLDAAFEKFKKDTLKPGEK

SEQ ID NO: 2 - protein, 79 aa, Streptococcus pneumoniae
KQVVDEYIEKMLREIQLDRRKHTQNVALNIKLSAIKTKYLRELNVLEEKSKDELPSEIKAKLDAAFEKFKKDTLKPGEK

SEQ ID NO: 3 - DNA, 2725 bp, Streptococcus pneumoniae
  misc_feature (2260)..(2260): n is a, c, g, or t
  misc_feature (2723)..(2723): n is a, c, g, or t
atgcttgtcaataatcacaaatatgtagatcatatcttgtttaggacagtaaaacatcctaattactttttaaatattcttcctgagttgattggcttgaccttgttgagtcatgcttatgtgacttttgttttagtttttccagtttatgcagttattttgtatcgacgaatagctgaagaggaaaagctattacatgaagttataatcccaaatggaagcataaagagataaatacaaaattcgatttatatacagttcatattgaagtaatatagtaaggttaaagaaaaaatatagaaggaaataaacatgtttgcatcaaaaagcgaaagaaaagtacattattcaattcgtaaatttagtattggagtagctagtgtagctgttgccagtcttgttatgggaagtgtggttcatgcgacagagaacgagggaagtacccaagcagccacttcttctaatatggcaaagacagaacataggaaagctgctaaacaagtcgtcgatgaatatatagaaaaaatgttgagggagattcaactagatagaagaaaacatacccaaaatgtcgccttaaacataaagttgagcgcaattaaaacgaagtatttgcgtgaattaaatgttttagaagagaagtcgaaagatgagttgccgtcagaaataaaagcaaagttagacgcagcttttgagaagtttaaaaaagatacattgaaaccaggagaaaaggtagcagaagctaagaagaaggttgaagaagctaagaaaaaagccgaggatcaaaaagaagaagatcgtcgtaactacccaaccaatacttacaaaacgcttgaacttgaaattgctgagttcgatgtgaaagttaaagaagcggagcttgaactagtaaaagaggaagctaaagaatctcgaaacgagggcacaattaagcaagcaaaagagaaagttgagagtaaaaaagctgaggctacaaggttagaaaacatcaagacagatcgtaaaaaagcagaagaagaagctaaacgaaaagcagatggtaagttgaaggaagctaatgtagcgacttcagatcaaggtaaaccaaaggggcgggcaaaacgaggagttcctggagagctagcaacacctgataaaaaagaaaatgatgcgaagtcttcagattctagcgtaggtgaagaaactcttccaagctcatccctgaaatcaggaaaaaaggtagcagaagctgagaagaaggttgaagaagctgagaaaaaagccaaggatcaaaaagaagaagatcgccgtaactacccaaccaatacttacaaaacgcttgaccttgaaattgctgagtccgatgtgaaagttaaagaagcggagcttgaactagtaaaagaggaagctaaggaacctcgagacgaggaaaaaattaagcaagcaaaagcgaaagttgagagtaaaaaagctgaggctacaaggttagaaaacatcaagacagatcgtaaaaaagcagaagaagaagctaaacgaaaagcagcagaagaagataaagttaaagaaaaaccagctgaacaaccacaaccagcgccggctactcaaccagaaaaaccagctccaaaaccagagaagccagctgaacaaccaaaagcagaaaaaacagatgatcaacaagctgaagaagactatgctcgtagatcagaagaagaatataatcgcttgactcaacagcaaccgccaaaaactgaaaaaccagcacaaccatctactccaaaaacaggctggaaacaagaaaacggtatgtggtacttctacaatactgatggttcaatggcaacaggatggctccaaaacaacggttcatggtactatctaaacgctaatggtgctatggcgacaggatggctccaaaacaatggttcatggtactatctaaacgctaatggttcaatggcaacaggatggctccaaaacaatggttcatggtactacctaaacgctaatggtgctatggcgacaggatggctccaatacaatggttcatggtactacctaaacagcaatggcgctatggcgacaggatggctccaatacaatggctcatggtactacctcaacgctaatggtgatatggcgacaggatggctccaaaacaacggttcatggtactacctcaacgctaatggtgatatggcgacaggatggctccaatacaacggttcatggtattacctcaacgctaatggtgatatggcgacaggttgggtgaaagatgganatacctggtactatcttaaagcatcaggtgctatgaaagcaagccaatggttcaaagtatcagataaatggtactatgtcaatggctcaggtgcccttgcagtcaacacaactgtagatggctatggagtcaatgccaatggtgaatgggtaaactaaacctaatataactagttaatactgacttcctgtaagaactttttaaagtattccctacaaataccatatcctttcagtagataatatacccttgtaggaagtttagattaaaaaataactctgtaatctctagccggatttatagcgctagagactacggagtttttttgatgaggaaagaatggcggcattcaagagactctttaagagagttacgggttttaaactattaagccttctccaattgcaagagggcttcaatctctgctagggtgctagcttgcgaaatggctccacggagtttngc

SEQ ID NO: 4 - protein, 701 aa, Streptococcus pneumoniae
  misc_feature (650)..(650): Xaa can be any naturally occurring amino acid
MFASKSERKVHYSIRKFSIGVASVAVASLVMGSVVHATENEGSTQAATSSNMAKTEHRKAAKQVVDEYIEKMLREIQLDRRKHTQNVALNIKLSAIKTKYLRELNVLEEKSKDELPSEIKAKLDAAFEKFKKDTLKPGEKVAEAKKKVEEAKKKAEDQKEEDRRNYPTNTYKTLELEIAEFDVKVKEAELELVKEEAKESRNEGTIKQAKEKVESKKAEATRLENIKTDRKKAEEEAKRKADGKLKEANVATSDQGKPKGRAKRGVPGELATPDKKENDAKSSDSSVGEETLPSSSLKSGKKVAEAEKKVEEAEKKAKDQKEEDRRNYPTNTYKTLDLEIAESDVKVKEAELELVKEEAKEPRDEEKIKQAKAKVESKKAEATRLENIKTDRKKAEEEAKRKAAEEDKVKEKPAEQPQPAPATQPEKPAPKPEKPAEQPKAEKTDDQQAEEDYARRSEEEYNRLTQQQPPKTEKPAQPSTPKTGWKQENGMWYFYNTDGSMATGWLQNNGSWYYLNANGAMATGWLQNNGSWYYLNANGSMATGWLQNNGSWYYLNANGAMATGWLQYNGSWYYLNSNGAMATGWLQYNGSWYYLNANGDMATGWLQNNGSWYYLNANGDMATGWLQYNGSWYYLNANGDMATGWVKDGXTWYYLKASGAMKASQWFKVSDKWYYVNGSGALAVNTTVDGYGVNANGEWVN

SEQ ID NO: 5 - DNA, 315 bp, Artificial Sequence
  codon-optimised DNA sequence used to express PspCN
gcaaccgaaaatgaaggtagcacccaggcagcaaccagcagcaatatggcaaaaaccgaacatcgtaaagcagccaaacaggttgtggatgagtatatcgaaaaaatgctgcgtgaaattcagctggatcgtcgtaaacatacccagaatgttgcactgaacattaaactgagcgccatcaaaaccaaatatctgcgtgaactgaatgtgctggaagagaaaagcaaagatgaactgccgagcgaaattaaagcaaaactggatgcagcctttgaaaaattcaaaaaagataccctgaaaccgggtgagaaataa

SEQ ID NO: 6 - protein, 1231 aa, Homo sapiens
MRLLAKIICLMLWAICVAEDCNELPPRRNTEILTGSWSDQTYPEGTQAIYKCRPGYRSLGNVIMVCRKGEWVALNPLRKCQKRPCGHPGDTPFGTFTLTGGNVFEYGVKAVYTCNEGYQLLGEINYRECDTDGWTNDIPICEVVKCLPVTAPENGKIVSSAMEPDREYHFGQAVRFVCNSGYKIEGDEEMHCSDDGFWSKEKPKCVEISCKSPDVINGSPISQKIIYKENERFQYKCNMGYEYSERGDAVCTESGWRPLPSCEEKSCDNPYIPNGDYSPLRIKHRTGDEITYQCRNGFYPATRGNTAKCTSTGWIPAPRCTLKPCDYPDIKHGGLYHENMRRPYFPVAVGKYYSYYCDEHFETPSGSYWDHIHCTQDGWSPAVPCLRKCYFPYLENGYNQNYGRKFVQGKSIDVACHPGYALPKAQTTVTCMENGWSPTPRCIRVKTCSKSSIDIENGFISESQYTYALKEKAKYQCKLGYVTADGETSGSITCGKDGWSAQPTCIKSCDIPVFMNARTKNDFTWFKLNDTLDYECHDGYESNTGSTTGSIVCGYNGWSDLPICYERECELPKIDVHLVPDRKKDQYKVGEVLKFSCKPGFTIVGPNSVQCYHFGLSPDLPICKEQVQSCGPPPELLNGNVKEKTKEEYGHSEVVEYYCNPRFLMKGPNKIQCVDGEWTTLPVCIVEESTCGDIPELEHGWAQLSSPPYYYGDSVEFNCSESFTMIGHRSITCIHGVWTQLPQCVAIDKLKKCKSSNLIILEEHLKNKKEFDHNSNIRYRCRGKEGWIHTVCINGRWDPEVNCSMAQIQLCPPPPQIPNSHNMTTTLNYRDGEKVSVLCQENYLIQEGEEITCKDGRWQSIPLCVEKIPCSQPPQIEHGTINSSRSSQESYAHGTKLSYTCEGGFRISEENETTCYMGKWSSPPQCEGLPCKSPPEISHGVVAHMSDSYQYGEEVTYKCFEGFGIDGPAIAKCLGEKWSHPPSCIKTDCLSLPSFENAIPMGEKKDVYKAGEQVTYTCATYYKMDGASNVTCINSRWTGRPTCRDTSCVNPPTVQNAYIVSRQMSKYPSGERVRYQCRSPYEMFGDEEVMCLNGNWTEPPQCKDSTGKCGPPPPIDNGDITSFPLSVYAPASSVEYQCQNLYQLEGNKRITCRNGQWSEPPKCLHPCVISREIMENYNIALRWTAKQKLYSRTGESVEFVCKRGYRLSSRSHTLRTTCWDGKLEYPTCAKR

SEQ ID NO: 7 - protein, 115 aa, Artificial Sequence
  N-terminally Cys modified PspCN
CGSGSGSGSGGATENEGSTQAATSSNMAKTEHRKAAKQVVDEYIEKMLREIQLDRRKHTQNVALNIKLSAIKTKYLRELNVLEEKSKDELPSEIKAKLDAAFEKFKKDTLKPGEK

SEQ ID NO: 8 - protein, 115 aa, Artificial Sequence
  C-terminally Cys modified PspCN
ATENEGSTQAATSSNMAKTEHRKAAKQVVDEYIEKMLREIQLDRRKHTQNVALNIKLSAIKTKYLRELNVLEEKSKDELPSEIKAKLDAAFEKFKKDTLKPGEKGSGSGSGSGGC

SEQ ID NO: 9 - protein, 143 aa, Streptococcus pneumoniae
ATENEGATQVPTSSNRANESQAEQGEQPKKLDSERDKARKEVEEYVKKIVGESYAKSTKKRHTITVALVNELNNIKNEYLNKIVESTSESQLQILMMESRSKVDEAVSKFEKDSSSSSSSDSSTKPEASDTAKPNKPTEPGEK